European Patent Application EP 4 293 042 A1, published December 20, 2023. Title: 一种TCR及其应用. Applicant: 深圳普瑞金生物药业有限公司. The sequence listing filed with the application follows.

SEQUENCE LISTING (74 sequences)

SEQ ID NO: 1 - protein, 9 aa, Homo sapiens
ASDQDARLM

SEQ ID NO: 2 - protein, 9 aa, Artificial Sequence
  A1 CDR3
AYDADARLM

SEQ ID NO: 3 - protein, 9 aa, Artificial Sequence
  A2 CDR3
AFDAHARLM

SEQ ID NO: 4 - protein, 9 aa, Artificial Sequence
  A3 CDR3
AYDEHARLM

SEQ ID NO: 5 - protein, 9 aa, Artificial Sequence
  A4 CDR3
AYDVHARLM

SEQ ID NO: 6 - protein, 9 aa, Artificial Sequence
  A5 CDR3
AYDQDARLM

SEQ ID NO: 7 - protein, 9 aa, Artificial Sequence
  A6 CDR3
AYDENARLM

SEQ ID NO: 8 - protein, 9 aa, Artificial Sequence
  A7 CDR3
AYDVAARLM

SEQ ID NO: 9 - protein, 9 aa, Artificial Sequence
  A8 CDR3
GYDQDARLM

SEQ ID NO: 10 - protein, 9 aa, Artificial Sequence
  A9 CDR3
SYDQEARLM

SEQ ID NO: 11 - protein, 9 aa, Artificial Sequence
  A10 CDR3
VYDQNARLM

SEQ ID NO: 12 - protein, 9 aa, Artificial Sequence
  A11 CDR3
AYDQWARLM

SEQ ID NO: 13 - protein, 10 aa, Homo sapiens
ASSLGPGELF

SEQ ID NO: 14 - protein, 10 aa, Artificial Sequence
  B1 CDR3
ASSLGANELF

SEQ ID NO: 15 - protein, 10 aa, Artificial Sequence
  B2 CDR3
ASSHGANELF

SEQ ID NO: 16 - protein, 10 aa, Artificial Sequence
  B3 CDR3
ASSLGSNELF

SEQ ID NO: 17 - protein, 10 aa, Artificial Sequence
  B4 CDR3
ASSRGSNELF

SEQ ID NO: 18 - protein, 109 aa, Homo sapiens
MSQQGEEDPQALSIQEGENATMNCSYKTSINNLQWYRQNSGRGLVHLILIRSNEREKHSGRLRVTLDTSKKSSSLLITASRAADTASYFCASDQDARLMFGDGTQLVVK

SEQ ID NO: 19 - protein, 109 aa, Artificial Sequence
  A1
MSQQGEEDPQALSIQEGENATMNCSYKTSINNLQWYRQNSGRGLVHLILIRSNEREKHSGRLRVTLDTSKKSSSLLITASRAADTASYFCAYDADARLMFGDGTQLVVK

SEQ ID NO: 20 - protein, 109 aa, Artificial Sequence
  A2
MSQQGEEDPQALSIQEGENATMNCSYKTSINNLQWYRQNSGRGLVHLILIRSNEREKHSGRLRVTLDTSKKSSSLLITASRAADTASYFCAFDAHARLMFGDGTQLVVK

SEQ ID NO: 21 - protein, 109 aa, Artificial Sequence
  A3
MSQQGEEDPQALSIQEGENATMNCSYKTSINNLQWYRQNSGRGLVHLILIRSNEREKHSGRLRVTLDTSKKSSSLLITASRAADTASYFCAYDEHARLMFGDGTQLVVK

SEQ ID NO: 22 - protein, 109 aa, Artificial Sequence
  A4
MSQQGEEDPQALSIQEGENATMNCSYKTSINNLQWYRQNSGRGLVHLILIRSNEREKHSGRLRVTLDTSKKSSSLLITASRAADTASYFCAYDVHARLMFGDGTQLVVK

SEQ ID NO: 23 - protein, 109 aa, Artificial Sequence
  A5
MSQQGEEDPQALSIQEGENATMNCSYKTSINNLQWYRQNSGRGLVHLILIRSNEREKHSGRLRVTLDTSKKSSSLLITASRAADTASYFCAYDQDARLMFGDGTQLVVK

SEQ ID NO: 24 - protein, 109 aa, Artificial Sequence
  A6
MSQQGEEDPQALSIQEGENATMNCSYKTSINNLQWYRQNSGRGLVHLILIRSNEREKHSGRLRVTLDTSKKSSSLLITASRAADTASYFCAYDENARLMFGDGTQLVVK

SEQ ID NO: 25 - protein, 109 aa, Artificial Sequence
  A7
MSQQGEEDPQALSIQEGENATMNCSYKTSINNLQWYRQNSGRGLVHLILIRSNEREKHSGRLRVTLDTSKKSSSLLITASRAADTASYFCAYDVAARLMFGDGTQLVVK

SEQ ID NO: 26 - protein, 109 aa, Artificial Sequence
  A8
MSQQGEEDPQALSIQEGENATMNCSYKTSINNLQWYRQNSGRGLVHLILIRSNEREKHSGRLRVTLDTSKKSSSLLITASRAADTASYFCGYDQDARLMFGDGTQLVVK

SEQ ID NO: 27 - protein, 109 aa, Artificial Sequence
  A9
MSQQGEEDPQALSIQEGENATMNCSYKTSINNLQWYRQNSGRGLVHLILIRSNEREKHSGRLRVTLDTSKKSSSLLITASRAADTASYFCSYDQEARLMFGDGTQLVVK

SEQ ID NO: 28 - protein, 109 aa, Artificial Sequence
  A10
MSQQGEEDPQALSIQEGENATMNCSYKTSINNLQWYRQNSGRGLVHLILIRSNEREKHSGRLRVTLDTSKKSSSLLITASRAADTASYFCVYDQNARLMFGDGTQLVVK

SEQ ID NO: 29 - protein, 109 aa, Artificial Sequence
  A11
MSQQGEEDPQALSIQEGENATMNCSYKTSINNLQWYRQNSGRGLVHLILIRSNEREKHSGRLRVTLDTSKKSSSLLITASRAADTASYFCAYDQWARLMFGDGTQLVVK

SEQ ID NO: 30 - protein, 109 aa, Artificial Sequence
  A0
MSQQGEEDPQALSIQEGENATINCSYKTSINNLQWYRQDPGRGLVHLILIRSNEREKHSGRLRVTLDTSKKSSSLEITATRPADTASYFCASDQDARLMFGDGTQLTVN

SEQ ID NO: 31 - protein, 109 aa, Artificial Sequence
  A1
MSQQGEEDPQALSIQEGENATINCSYKTSINNLQWYRQDPGRGLVHLILIRSNEREKHSGRLRVTLDTSKKSSSLEITATRPADTASYFCAYDADARLMFGDGTQLTVN

SEQ ID NO: 32 - protein, 109 aa, Artificial Sequence
  A2
MSQQGEEDPQALSIQEGENATINCSYKTSINNLQWYRQDPGRGLVHLILIRSNEREKHSGRLRVTLDTSKKSSSLEITATRPADTASYFCAFDAHARLMFGDGTQLTVN

SEQ ID NO: 33 - protein, 109 aa, Artificial Sequence
  A3
MSQQGEEDPQALSIQEGENATINCSYKTSINNLQWYRQDPGRGLVHLILIRSNEREKHSGRLRVTLDTSKKSSSLEITATRPADTASYFCAYDEHARLMFGDGTQLTVN

SEQ ID NO: 34 - protein, 109 aa, Artificial Sequence
  A4
MSQQGEEDPQALSIQEGENATINCSYKTSINNLQWYRQDPGRGLVHLILIRSNEREKHSGRLRVTLDTSKKSSSLEITATRPADTASYFCAYDVHARLMFGDGTQLTVN

SEQ ID NO: 35 - protein, 109 aa, Artificial Sequence
  A5
MSQQGEEDPQALSIQEGENATINCSYKTSINNLQWYRQDPGRGLVHLILIRSNEREKHSGRLRVTLDTSKKSSSLEITATRPADTASYFCAYDQDARLMFGDGTQLTVN

SEQ ID NO: 36 - protein, 109 aa, Artificial Sequence
  A6
MSQQGEEDPQALSIQEGENATINCSYKTSINNLQWYRQDPGRGLVHLILIRSNEREKHSGRLRVTLDTSKKSSSLEITATRPADTASYFCAYDENARLMFGDGTQLTVN

SEQ ID NO: 37 - protein, 109 aa, Artificial Sequence
  A7
MSQQGEEDPQALSIQEGENATINCSYKTSINNLQWYRQDPGRGLVHLILIRSNEREKHSGRLRVTLDTSKKSSSLEITATRPADTASYFCAYDVAARLMFGDGTQLTVN

SEQ ID NO: 38 - protein, 109 aa, Artificial Sequence
  A8
MSQQGEEDPQALSIQEGENATINCSYKTSINNLQWYRQDPGRGLVHLILIRSNEREKHSGRLRVTLDTSKKSSSLEITATRPADTASYFCGYDQDARLMFGDGTQLTVN

SEQ ID NO: 39 - protein, 109 aa, Artificial Sequence
  A9
MSQQGEEDPQALSIQEGENATINCSYKTSINNLQWYRQDPGRGLVHLILIRSNEREKHSGRLRVTLDTSKKSSSLEITATRPADTASYFCSYDQEARLMFGDGTQLTVN

SEQ ID NO: 40 - protein, 109 aa, Artificial Sequence
  A10
MSQQGEEDPQALSIQEGENATINCSYKTSINNLQWYRQDPGRGLVHLILIRSNEREKHSGRLRVTLDTSKKSSSLEITATRPADTASYFCVYDQNARLMFGDGTQLTVN

SEQ ID NO: 41 - protein, 109 aa, Artificial Sequence
  A11
MSQQGEEDPQALSIQEGENATINCSYKTSINNLQWYRQDPGRGLVHLILIRSNEREKHSGRLRVTLDTSKKSSSLEITATRPADTASYFCAYDQWARLMFGDGTQLTVN

SEQ ID NO: 42 - protein, 112 aa, Homo sapiens
DAGVIQSPRHEVTEMGQEVTLRCKPISGHDYLFWYRQTMMRGLELLIYFNNNVPIDDSGMPEDRFSAKMPNASFSTLKIQPSEPRDSAVYFCASSLGPGELFFGEGSRLTVL

SEQ ID NO: 43 - protein, 112 aa, Artificial Sequence
  B1
DAGVIQSPRHEVTEMGQEVTLRCKPISGHDYLFWYRQTMMRGLELLIYFNNNVPIDDSGMPEDRFSAKMPNASFSTLKIQPSEPRDSAVYFCASSLGANELFFGEGSRLTVL

SEQ ID NO: 44 - protein, 112 aa, Artificial Sequence
  B2
DAGVIQSPRHEVTEMGQEVTLRCKPISGHDYLFWYRQTMMRGLELLIYFNNNVPIDDSGMPEDRFSAKMPNASFSTLKIQPSEPRDSAVYFCASSHGANELFFGEGSRLTVL

SEQ ID NO: 45 - protein, 112 aa, Artificial Sequence
  B3
DAGVIQSPRHEVTEMGQEVTLRCKPISGHDYLFWYRQTMMRGLELLIYFNNNVPIDDSGMPEDRFSAKMPNASFSTLKIQPSEPRDSAVYFCASSLGSNELFFGEGSRLTVL

SEQ ID NO: 46 - protein, 112 aa, Artificial Sequence
  B4
DAGVIQSPRHEVTEMGQEVTLRCKPISGHDYLFWYRQTMMRGLELLIYFNNNVPIDDSGMPEDRFSAKMPNASFSTLKIQPSEPRDSAVYFCASSRGSNELFFGEGSRLTVL

SEQ ID NO: 47 - protein, 112 aa, Artificial Sequence
  B0
DAGVTQSPRHITVPQGQEVTLRCKPISGHDYLFWYRQDPGRGLELLIYFNNNVPIDDSGMPEDRFSAKMPNASHSTLKIQPSEPRDSAVYFCASSLGPGELFFGEGSRLTVN

SEQ ID NO: 48 - protein, 112 aa, Artificial Sequence
  B1
DAGVTQSPRHITVPQGQEVTLRCKPISGHDYLFWYRQDPGRGLELLIYFNNNVPIDDSGMPEDRFSAKMPNASHSTLKIQPSEPRDSAVYFCASSLGANELFFGEGSRLTVN

SEQ ID NO: 49 - protein, 112 aa, Artificial Sequence
  B2
DAGVTQSPRHITVPQGQEVTLRCKPISGHDYLFWYRQDPGRGLELLIYFNNNVPIDDSGMPEDRFSAKMPNASHSTLKIQPSEPRDSAVYFCASSHGANELFFGEGSRLTVN

SEQ ID NO: 50 - protein, 112 aa, Artificial Sequence
  B3
DAGVTQSPRHITVPQGQEVTLRCKPISGHDYLFWYRQDPGRGLELLIYFNNNVPIDDSGMPEDRFSAKMPNASHSTLKIQPSEPRDSAVYFCASSLGSNELFFGEGSRLTVN

SEQ ID NO: 51 - protein, 112 aa, Artificial Sequence
  B4
DAGVTQSPRHITVPQGQEVTLRCKPISGHDYLFWYRQDPGRGLELLIYFNNNVPIDDSGMPEDRFSAKMPNASHSTLKIQPSEPRDSAVYFCASSRGSNELFFGEGSRLTVN

SEQ ID NO: 52 - protein, 270 aa, Homo sapiens
METLLGVSLVILWLQLARVNSQQGEEDPQALSIQEGENATMNCSYKTSINNLQWYRQNSGRGLVHLILIRSNEREKHSGRLRVTLDTSKKSSSLLITASRAADTASYFCASDQDARLMFGDGTQLVVKPNIQNPDPAVYQLRDSKSSDKSVCLFTDFDSQTNVSQSKDSDVYITDKTVLDMRSMDFKSNSAVAWSNKSDFACANAFNNSIIPEDTFFPSPESSCDVKLVEKSFETDTNLNFQNLSVIGFRILLLKVAGFNLLMTLRLWSS

SEQ ID NO: 53 - protein, 310 aa, Homo sapiens
MDSWTLCCVSLCILVAKHTDAGVIQSPRHEVTEMGQEVTLRCKPISGHDYLFWYRQTMMRGLELLIYFNNNVPIDDSGMPEDRFSAKMPNASFSTLKIQPSEPRDSAVYFCASSLGPGELFFGEGSRLTVLEDLKNVFPPEVAVFEPSEAEISHTQKATLVCLATGFYPDHVELSWWVNGKEVHSGVSTDPQPLKEQPALNDSRYCLSSRLRVSATFWQNPRNHFRCQVQFYGLSENDEWTQDRAKPVTQIVSAEAWGRADCGFTSESYQQGVLSATILYEILLGKATLYAVLVSALVLMAMVKRKDSRG

SEQ ID NO: 54 - protein, 221 aa, Homo sapiens
MSQQGEEDPQALSIQEGENATMNCSYKTSINNLQWYRQNSGRGLVHLILIRSNEREKHSGRLRVTLDTSKKSSSLLITASRAADTASYFCASDQDARLMFGDGTQLVVKPNIQNPDPAVYQLRDSKSSDKSVCLFTDFDSQTNVSQSKDSDVYITDKTVLDMRSMDFKSNSAVAWSNKSDFACANAFNNSIIPEDTFFPSPESSCDVKLVEKSFETDTNLN

SEQ ID NO: 55 - protein, 221 aa, Artificial Sequence
  A1
MSQQGEEDPQALSIQEGENATMNCSYKTSINNLQWYRQNSGRGLVHLILIRSNEREKHSGRLRVTLDTSKKSSSLLITASRAADTASYFCAYDADARLMFGDGTQLVVKPNIQNPDPAVYQLRDSKSSDKSVCLFTDFDSQTNVSQSKDSDVYITDKTVLDMRSMDFKSNSAVAWSNKSDFACANAFNNSIIPEDTFFPSPESSCDVKLVEKSFETDTNLN

SEQ ID NO: 56 - protein, 221 aa, Artificial Sequence
  A2
MSQQGEEDPQALSIQEGENATMNCSYKTSINNLQWYRQNSGRGLVHLILIRSNEREKHSGRLRVTLDTSKKSSSLLITASRAADTASYFCAFDAHARLMFGDGTQLVVKPNIQNPDPAVYQLRDSKSSDKSVCLFTDFDSQTNVSQSKDSDVYITDKTVLDMRSMDFKSNSAVAWSNKSDFACANAFNNSIIPEDTFFPSPESSCDVKLVEKSFETDTNLN

SEQ ID NO: 57 - protein, 221 aa, Artificial Sequence
  A3
MSQQGEEDPQALSIQEGENATMNCSYKTSINNLQWYRQNSGRGLVHLILIRSNEREKHSGRLRVTLDTSKKSSSLLITASRAADTASYFCAYDEHARLMFGDGTQLVVKPNIQNPDPAVYQLRDSKSSDKSVCLFTDFDSQTNVSQSKDSDVYITDKTVLDMRSMDFKSNSAVAWSNKSDFACANAFNNSIIPEDTFFPSPESSCDVKLVEKSFETDTNLN

SEQ ID NO: 58 - protein, 221 aa, Artificial Sequence
  A4
MSQQGEEDPQALSIQEGENATMNCSYKTSINNLQWYRQNSGRGLVHLILIRSNEREKHSGRLRVTLDTSKKSSSLLITASRAADTASYFCAYDVHARLMFGDGTQLVVKPNIQNPDPAVYQLRDSKSSDKSVCLFTDFDSQTNVSQSKDSDVYITDKTVLDMRSMDFKSNSAVAWSNKSDFACANAFNNSIIPEDTFFPSPESSCDVKLVEKSFETDTNLN

SEQ ID NO: 59 - protein, 221 aa, Artificial Sequence
  A5
MSQQGEEDPQALSIQEGENATMNCSYKTSINNLQWYRQNSGRGLVHLILIRSNEREKHSGRLRVTLDTSKKSSSLLITASRAADTASYFCAYDQDARLMFGDGTQLVVKPNIQNPDPAVYQLRDSKSSDKSVCLFTDFDSQTNVSQSKDSDVYITDKTVLDMRSMDFKSNSAVAWSNKSDFACANAFNNSIIPEDTFFPSPESSCDVKLVEKSFETDTNLN

SEQ ID NO: 60 - protein, 221 aa, Artificial Sequence
  A6
MSQQGEEDPQALSIQEGENATMNCSYKTSINNLQWYRQNSGRGLVHLILIRSNEREKHSGRLRVTLDTSKKSSSLLITASRAADTASYFCAYDENARLMFGDGTQLVVKPNIQNPDPAVYQLRDSKSSDKSVCLFTDFDSQTNVSQSKDSDVYITDKTVLDMRSMDFKSNSAVAWSNKSDFACANAFNNSIIPEDTFFPSPESSCDVKLVEKSFETDTNLN

SEQ ID NO: 61 - protein, 221 aa, Artificial Sequence
  A7
MSQQGEEDPQALSIQEGENATMNCSYKTSINNLQWYRQNSGRGLVHLILIRSNEREKHSGRLRVTLDTSKKSSSLLITASRAADTASYFCAYDVAARLMFGDGTQLVVKPNIQNPDPAVYQLRDSKSSDKSVCLFTDFDSQTNVSQSKDSDVYITDKTVLDMRSMDFKSNSAVAWSNKSDFACANAFNNSIIPEDTFFPSPESSCDVKLVEKSFETDTNLN

SEQ ID NO: 62 - protein, 221 aa, Artificial Sequence
  A8
MSQQGEEDPQALSIQEGENATMNCSYKTSINNLQWYRQNSGRGLVHLILIRSNEREKHSGRLRVTLDTSKKSSSLLITASRAADTASYFCGYDQDARLMFGDGTQLVVKPNIQNPDPAVYQLRDSKSSDKSVCLFTDFDSQTNVSQSKDSDVYITDKTVLDMRSMDFKSNSAVAWSNKSDFACANAFNNSIIPEDTFFPSPESSCDVKLVEKSFETDTNLN

SEQ ID NO: 63 - protein, 221 aa, Artificial Sequence
  A9
MSQQGEEDPQALSIQEGENATMNCSYKTSINNLQWYRQNSGRGLVHLILIRSNEREKHSGRLRVTLDTSKKSSSLLITASRAADTASYFCSYDQEARLMFGDGTQLVVKPNIQNPDPAVYQLRDSKSSDKSVCLFTDFDSQTNVSQSKDSDVYITDKTVLDMRSMDFKSNSAVAWSNKSDFACANAFNNSIIPEDTFFPSPESSCDVKLVEKSFETDTNLN

SEQ ID NO: 64 - protein, 221 aa, Artificial Sequence
  A10
MSQQGEEDPQALSIQEGENATMNCSYKTSINNLQWYRQNSGRGLVHLILIRSNEREKHSGRLRVTLDTSKKSSSLLITASRAADTASYFCVYDQNARLMFGDGTQLVVKPNIQNPDPAVYQLRDSKSSDKSVCLFTDFDSQTNVSQSKDSDVYITDKTVLDMRSMDFKSNSAVAWSNKSDFACANAFNNSIIPEDTFFPSPESSCDVKLVEKSFETDTNLN

SEQ ID NO: 65 - protein, 221 aa, Artificial Sequence
  A11
MSQQGEEDPQALSIQEGENATMNCSYKTSINNLQWYRQNSGRGLVHLILIRSNEREKHSGRLRVTLDTSKKSSSLLITASRAADTASYFCAYDQWARLMFGDGTQLVVKPNIQNPDPAVYQLRDSKSSDKSVCLFTDFDSQTNVSQSKDSDVYITDKTVLDMRSMDFKSNSAVAWSNKSDFACANAFNNSIIPEDTFFPSPESSCDVKLVEKSFETDTNLN

SEQ ID NO: 66 - protein, 259 aa, Homo sapiens
MDAGVIQSPRHEVTEMGQEVTLRCKPISGHDYLFWYRQTMMRGLELLIYFNNNVPIDDSGMPEDRFSAKMPNASFSTLKIQPSEPRDSAVYFCASSLGPGELFFGEGSRLTVLEDLKNVFPPEVAVFEPSEAEISHTQKATLVCLATGFYPDHVELSWWVNGKEVHSGVSTDPQPLKEQPALNDSRYCLSSRLRVSATFWQNPRNHFRCQVQFYGLSENDEWTQDRAKPVTQIVSAEAWGRADCGFTSESYQQGVLSAT

SEQ ID NO: 67 - protein, 259 aa, Artificial Sequence
  B1
MDAGVIQSPRHEVTEMGQEVTLRCKPISGHDYLFWYRQTMMRGLELLIYFNNNVPIDDSGMPEDRFSAKMPNASFSTLKIQPSEPRDSAVYFCASSLGANELFFGEGSRLTVLEDLKNVFPPEVAVFEPSEAEISHTQKATLVCLATGFYPDHVELSWWVNGKEVHSGVSTDPQPLKEQPALNDSRYCLSSRLRVSATFWQNPRNHFRCQVQFYGLSENDEWTQDRAKPVTQIVSAEAWGRADCGFTSESYQQGVLSAT

SEQ ID NO: 68 - protein, 259 aa, Artificial Sequence
  B2
MDAGVIQSPRHEVTEMGQEVTLRCKPISGHDYLFWYRQTMMRGLELLIYFNNNVPIDDSGMPEDRFSAKMPNASFSTLKIQPSEPRDSAVYFCASSHGANELFFGEGSRLTVLEDLKNVFPPEVAVFEPSEAEISHTQKATLVCLATGFYPDHVELSWWVNGKEVHSGVSTDPQPLKEQPALNDSRYCLSSRLRVSATFWQNPRNHFRCQVQFYGLSENDEWTQDRAKPVTQIVSAEAWGRADCGFTSESYQQGVLSAT

SEQ ID NO: 69 - protein, 259 aa, Artificial Sequence
  B3
MDAGVIQSPRHEVTEMGQEVTLRCKPISGHDYLFWYRQTMMRGLELLIYFNNNVPIDDSGMPEDRFSAKMPNASFSTLKIQPSEPRDSAVYFCASSLGSNELFFGEGSRLTVLEDLKNVFPPEVAVFEPSEAEISHTQKATLVCLATGFYPDHVELSWWVNGKEVHSGVSTDPQPLKEQPALNDSRYCLSSRLRVSATFWQNPRNHFRCQVQFYGLSENDEWTQDRAKPVTQIVSAEAWGRADCGFTSESYQQGVLSAT

SEQ ID NO: 70 - protein, 259 aa, Artificial Sequence
  B4
MDAGVIQSPRHEVTEMGQEVTLRCKPISGHDYLFWYRQTMMRGLELLIYFNNNVPIDDSGMPEDRFSAKMPNASFSTLKIQPSEPRDSAVYFCASSRGSNELFFGEGSRLTVLEDLKNVFPPEVAVFEPSEAEISHTQKATLVCLATGFYPDHVELSWWVNGKEVHSGVSTDPQPLKEQPALNDSRYCLSSRLRVSATFWQNPRNHFRCQVQFYGLSENDEWTQDRAKPVTQIVSAEAWGRADCGFTSESYQQGVLSAT

SEQ ID NO: 71 - protein, 5 aa, Homo sapiens
TSINN

SEQ ID NO: 72 - protein, 7 aa, Homo sapiens
IRSNERE

SEQ ID NO: 73 - protein, 5 aa, Homo sapiens
SGHDY

SEQ ID NO: 74 - protein, 6 aa, Homo sapiens
FNNNVP